European Patent Specification EP 3 897 727 B1, published May 15, 2024. Title: TREATMENT of CANCER HARBORING MUTATIONS in the TP53 GENE and/or POST- TRANSLATIONAL MODIFICATIONS in the P53 PROTEIN with PARVOVIRUSES. Applicant: UNIVERSIDAD AUTÓNOMA DE MADRID. The sequence listing filed with the application follows.

SEQUENCE LISTING (20 sequences)

SEQ ID NO: 1 - DNA, 5149 bp, Parvovirus diminuto de ratón MVMp
atttttagaactgaccaaccatgttcacgtaagtgacgtgatgacgcgcgctgcgcgcgcgccttcggacgtcacacgtcacttacgtttcacatggttggtcagttctaaaaatgataagcggttcagggagtttaaaccaaggcgcgaaaaggaagtgggcgtggtttaaagtatataagcaactactgaagtcagttacttatcttttctttcattctgtgagtcgagacgcacagaaagagagtaaccaactaaccatggctggaaatgcttactctgatgaagttttgggagcaaccaactggttaaaggaaaaaagtaaccaggaagtgttctcatttgtttttaaaaatgaaaatgttcaactgaatggaaaagatatcggatggaatagttacaaaaaagagctgcaggaggacgagctgaaatctttacaacgaggagcggaaactacttgggaccaaagcgaggacatggaatgggaaaccacagtggatgaaatgaccaaaaagcaagtattcatttttgattctttggttaaaaaatgtttatttgaagtgcttaacacaaagaatatatttcctggtgatgttaattggtttgtgcaacatgaatggggaaaagaccaaggctggcactgccatgtactaattggaggaaaggactttagtcaagctcaagggaaatggtggagaaggcaactaaatgtttactggagcagatggttggtaacagcctgtaatgtgcaactaacaccagctgaaagaattaaactaagagaaatagcagaagacaatgagtgggttactctacttacttataagcataagcaaaccaaaaaagactataccaagtgtgttctttttggaaacatgattgcttactattttttaactaaaaagaaaataagcactagtccaccaagagacggaggctattttcttagcagtgactctggctggaaaactaactttttaaaagaaggcgagcgccatctagtgagcaaactatacactgatgacatgcggccagaaacggttgaaaccacagtaaccactgcgcaggaaactaagcgcggcagaattcaaactaaaaaagaagtttctattaaaactacacttaaagagctggtgcataaaagagtaacctcaccagaggactggatgatgatgcagccagacagttacattgaaatgatggctcaaccaggtggagaaaacctgctgaaaaatacgctagagatttgtacactaactctagccagaaccaaaacagcatttgacttaattttagaaaaagctgaaaccagcaaactaaccaacttttcactgcctgacacaagaacctgcagaatttttgcttttcatggctggaactatgttaaagtttgccatgctatttgctgtgttttaaacagacaaggaggcaaaagaaatactgttttatttcatggaccagccagcacaggcaaatctattattgcacaagccatagcacaagcagttggcaatgttggttgctataatgcagccaatgtaaactttccatttaatgactgtaccaacaagaacttgatttgggtagaagaagctggtaactttggacagcaagtaaaccagtttaaagccatttgctctggtcaaactattcgcattgatcaaaaaggaaaaggcagcaaacagattgaaccaacaccagtcatcatgaccacaaatgagaacattacagtggtcagaataggctgcgaagaaagaccagaacacactcaaccaatcagagacagaatgcttaacattcatctaacacataccttgcctggtgactttggtttggttgacaaaaatgaatggcccatgatttgtgcttggttggtaaagaatggttaccaatctaccatggcaagctactgtgctaaatggggcaaagttcctgattggtcagaaaactgggcggagccaaaggtgccaactcctataaatttactaggttcggcacgctcaccattcacgacaccgaaaagtacgcctctcagccagaactatgcactaactccacttgcatcggatctcgaggacctggctttagagccttggagcacaccaaatactcctgttgcgggcactgcagaaacccagaacactggggaagctggttccaaagcctgccaagatggtcaactgagcccaacttggtcagagatcgaggaggatttgagagcgtgcttcggtgcggaaccgttgaagaaagacttcagcgagccgctgaacttggactaaggtacgatggcgcctccagctaaaagagctaaaagaggtaagggtttaagggatggttggttggtggggtattaatgtttaattacctgttttacaggcctgaaatcacttggttttaggttgggtgcctcctggctacaagtacctgggaccagggaacagccttgaccaaggagaaccaaccaatccatctgacgccgctgccaaagagcacgacgaggcctatgatcaatacatcaaatctggaaaaaatccttacctgtacttctctgctgctgatcaacgctttattgaccaaaccaaggacgccaaagactggggaggcaaggttggtcactacttttttagaaccaagcgcgcttttgcacctaagcttgctactgactctgaacctggaacttctggtgtaagcagagctggtaaacgcactagaccacctgcttacatttttattaaccaagccagagctaaaaaaaaacttacttcttctgctgcacagcaaagcagtcaaaccatgagtgatggcaccagccaacctgacagcggaaacgctgtccactcagctgcaagagttgaacgagcagctgacggccctggaggctctgggggtgggggctctggcgggggtggggttggtgtttctactgggtcttatgataatcaaacgcattatagattcttgggtgacggctgggtagaaattactgcactagcaactagactagtacatttaaacatgcctaaatcagaaaactattgcagaatcagagttcacaatacaacagacacatcagtcaaaggcaacatggcaaaagatgatgctcatgagcaaatttggacaccatggagcttggtggatgctaatgcttggggagtttggctccagccaagtgactggcaatacatttgcaacaccatgagccagcttaacttggtatcacttgatcaagaaatattcaatgtagtgctgaaaactgttacagagcaagacttaggaggtcaagctataaaaatatacaacaatgaccttacagcttgcatgatggttgcagtagactcaaacaacattttgccatacacacctgcagcaaactcaatggaaacacttggtttctacccctggaaaccaaccatagcatcaccatacaggtactatttttgcgttgacagagatctttcagtgacctacgaaaatcaagaaggcacagttgaacataatgtgatgggaacaccaaaaggaatgaattctcaattttttaccattgagaacacacaacaaatcacattgctcagaacaggggacgaatttgccacaggtacttactactttgacacaaattcagttaaactcacacacacgtggcaaaccaaccgtcaacttggacagcctccactgctgtcaacctttcctgaagctgacactgatgcaggtacacttactgctcaagggagcagacatggaacaacacaaatgggggttaactgggtgagtgaagcaatcagaaccagacctgctcaagtaggattttgtcaaccacacaatgactttgaagccagcagagctggaccatttgctgccccaaaagttccagcagatattactcaaggagtagacaaagaagccaatggcagtgttagatacagttatggcaaacagcatggtgaaaattgggcttcacatggaccagcaccagagcgctacacatgggatgaaacaagctttggttcaggtagagacaccaaagatggttttattcaatcagcaccactagttgttccaccaccactaaatggcattcttacaaatgcaaaccctattgggactaaaaatgacattcatttttcaaatgtttttaacagctatggtccactaactgcattttcacacccaagtcctgtataccctcaaggacaaatatgggacaaagaactagatcttgaacacaaacctagacttcacataactgctccatttgtttgtaaaaacaatgcacctggacaaatgttggttagattaggaccaaacctaactgaccaatatgatccaaacggagccacactttctagaattgttacatacggtacatttttctggaaaggaaaactaaccatgagagcaaaacttagagctaacaccacttggaacccagtgtaccaagtaagtgctgaagacaatggcaactcatacatgagtgtaactaaatggttaccaactgctactggaaacatgcagtctgtgccgcttataacaagacctgttgctagaaatacttactaactaaccatgctttttctttctgtacttcatatattattaagactaataaagatacaacatagaaatataatattacgtatagatttaagaaatagaataatatggtacttagtaactgttaaaaataatagaacctttggaataacaagatagttagttggttaatgttagatagaataagaagatcatgtataatgaataaaagggtggaagggtggttggtaggttaatgttagatagaataagaagatcatgtataatgaataaaagggtggaagggtggttggtaggtattcccttagacttgatgttaaggaccaaaaaaataataaaacttttttaaaactcaaccaagactactgtctattcagtgaaccaactgaaccattagtattactatgtttttagggtgggagggtgggagatacatgtgttcgctatgagcgaactggtactggttggttgctctgctcaaccaaccagaccggcaaagccggtctggttggttgagcgcaaccaaccagtaccagttcgctcatagcgaacacatgtatctcccaccctcccaccctaaaaacatagtaatactaat

SEQ ID NO: 2 - DNA, 5087 bp, Parvovirus diminuto de ratón MVMi
atttttagaactgaccaaccatgttcacgtaagtgacgtgatgacgcgcgcttcgcgcgctgcctgcggcagtcacacgtcacttacgtctcacatggttggtcagttctaaaaatgataagcggttcagagagtttagaccaaggcgcgaaaaggaagtgggcgtggtttaaagtatataagcaaatgctgaagtcagttacttatcctttctttcattctgtgagtcgagacgcgcagaaagagagtaaccaactaaccatggctggaaatgcttactctgatgaagttttgggaacaaccaactggttaaaggaaaaaagtaaccaggaagtgttctcatttgtttttaaaactgaggatgttcaactaaatggaaaagatatcggatggaataattacaaaaaggagctgcaggaggacgagctgaaatctttacaacgaggagcggaaactacctgggaccaaagcgaggacatggaatgggaatctacagtggatgaaatgaccaaaaagcaagtattcatttatgactctttagttaaaaaatgtttgtttgaagtgcttagcacaaaaaatatagctcctgctgatgttacttggtttgtgcagcatgaatgggggaaagaccaaggctggcactgccatgtactaattggaggcaaggactttagtcaagctcaaggaaaatggtggagaaggcagctaaatgtttactggagcagatggttggtaacagcctgtaatgtgcagctaacaccagctgaaagaattaaactaagagaaatagcagaagacagtgagtgggttactttactcacttataaacataagcaaaccaaaaaggactatactaaatgtgttctttttggaaatatgattgcttactactttttaaccaaaaagaaaataagcaccagtccgccaagggacggaggctattttctaagcagtgactctggctggaaaactaactttttaaaagagggcgaacgccatctagtgagcaaattatacactgatgacatgcggccagaaacggttgaaaccacagtaaccactgcgcaggaaactaagcgcggcagaattcaaactaaaaaagaggtttctattaaaaccacacttaaagagctagtgcataaaagagtaacctcaccagaagactggatgatgatgcagccagacagttacattgaaatgatggctcaaccaggtggagaaaacctgctgaaaaatacgctagagatttgtacgctaactctagccagaacaaaaacagcatttgacttgattttagaaaaagctgaaaccagcaaactaaccaacttttcactgcctgacacaagaacctgcaagatttttgcttttcatggctggaactatgttaaagtttgccatgctatttgctgtgttctaaacagacaaggaggcaaaagaaatactgttttatttcacggaccagccagtacaggcaaatctattattgcacaagccatagcacaggcagttggtaatgttggttgctataatgcagctaatgtgaactttccatttaatgactgtacgaacaaaaacttgatttgggtagaagaagctggtaactttggacagcaagtaaaccagtttaaagccatttgctctggtcaaactattcgcattgatcaaaaaggaaaaggcagcaaacaaattgaaccaacaccagtcatcatgaccacaaatgagaacattacagtggtcagaataggctgcgaagagagaccagaacacactcaaccaattagagacagaatgctcaacattcatctaacacatacattgcctggtgactttggtttggttgacaagaatgaatggcccatgatttgtgcttggttggtaaagaatggttaccaatctaccatggcaagctactgcgctaaatggggcaaagttcctgattggtcagaaaactgggcggagccgaaggtgccgactcctataaattcactaggttcggcacgctcaccattcacgacaccgaaaagtacgcctctcagccagaactatgcactaactccacttgcatcggatctcgaggacctggctttagagccttggagcacaccaaatactcctgttgcgggcactgcagaaacccagaacactggggaagctggttccaaagcctgccaagatggtcaactgagcccaacttggtcagagatcgaggaggatttgagagcgtgcttcggtgcggaaccgttgaagagagacttcagcgagccgctgaacttggactaaggtacgatggcgcctccagctaaaagagctaaaagaggtaagggtttaagggatggttggttggtggggtattaatgtttaattacctgttttacaggcctgaaatcacttggttttaggttgggtgcctcctggctataagtacctgggaccagggaacagccttgaccaaggagaaccaaccaatccatctgacgccgctgccaaagagcacgacgaggcctatgatcaatacatcaaatctggaaaaaatccttacctgtacttctctgctgctgatcaacgctttattgaccaaaccaaggacgccaaagactggggaggcaaggttggtcactacttttttagaaccaagcgcgcttttgcacctaagcttgctactgactctgaacctggaacttctggtgtaagcagagctggtaaacgcactagaccacctgcttacatttttataaaccaagccagagctaaaaaaaaacttacttcttctgctgcacagcaaagcagtcaaaccatgagtgatggcaccagccaacctgacggcggaaacggtgtccactcagctgcaagagttgaacgagcagctgacggccctggaggctctgggggtgggggctctggcgggggtggggttggtgtttctactgggtcttatgataatcagacgcattatagattcttgggtgacggctgggtagaaattactgcactagcaactagactagtacatttaaacatgcctaaatcagaaaactattgcagaataagagttcacaacacaacagacacttcagtcaaaggcaacatggcaaaagatgatgctcatgagcaaatttggacgccatggagcttagtggatgctaatgcttggggagtttggctccagccaagtgactggcaatacatttgcaacaccatgagccagcttaacttggtctcacttgatcaagaaatatttaatgtagtgctgaaaactgttacagagcaagactcaggaggtcaagctataaaaatatacaacaatgacctcacagcttgcatgatggttgcagtagactcaaacaacattctgccatacacacctgcagcaaactcaatggaaacacttggtttctacccttggaaaccaactatagcatcgccatacaggtactatttctgcgttgacagagatctttcagtaacctatgaaaatcaagaaggcacaattgagcataatgtaatgggaacaccaaaaggaatgaattctcaattttttaccattgagaacacacaacaaatcacattgctcagaactggtgatgagtttgctactggaacctactactttgacacaaacccagttaaacttacacacacatggcaaactaaccgtcaacttggacagcctccactgctgtcaacctttcctgaagctgacactgatgcaggtacacttactgctcaagggagcagacatggagcaacacagatggaggttaactgggtgagtgaagcaattagaaccagacctgctcaagtaggattttgtcagccacacaatgactttgaagccagcagagctggaccatttgctgctccaaaagttccagcagatgttactcaaggagtggacagagaagccaatggcagtgttagatacagttatggcaaacagcatggtgaaaattgggctgcacacggaccagcaccagagcgctacacatgggatgaaacaaactttggttcaggaagagacaccagagatggttttattcaatcagcacctctagttgttccaccaccactaaatgggattcttacaaatgcaaaccctattggaactaaaaatgacattcatttttcaaatgtttttaacagctatggtccactaactgcattttcacacccaagtcctgtataccctcaaggacaaatatgggacaaagaactagatcttgaacacaaacctagacttcacataactgctccatttgtctgtaaaaacaatgcacctggacaaatgttggttagattaggaccaaatctaactgaccagtatgatccaaacggagccacactttctagaattgtgacttatggtacatttttctggaaaggaaaactaacaatgagagcaaaacttagagctaacaccacttggaacccagtgtaccaagtaagtgttgaagacaatggcaactcatacatgagtgttactaaatggctaccaactgctactggaaacatgcaatctgtaccgcttataacaagacctgttgctagaaatacttactaactaaccatgtttttcctttctgtacttcatatattattaagactaataaagatacaacataaaaatataatattacatatagatttaagaaatagaataatatggtacttagtaactgttagaaataatagaacctttggaataacaagataattagttggttaatgttagatagaataagaagattatgtataatgggtaaaagggtggaagggtggttggttggtattcccttagacatgatgttaaggaccaaaaaaataataaaattttttaaaactaaaccaagactactgtctattcagttgaaccaactgaaccatcagtatcactatgtttttagggtgggggggtgggagatacatgtgttcgctatgagcgaactggtactggttggttgctctgctcaaccaaccagaccggctttgccggtctggttggttgagcgcaaccaaccagtaccagttcgctcatagcgaacacatgtatctcccacccccccaccctaaaaacatagtgatactgatgg

SEQ ID NO: 3 - DNA, 5135 bp, Parvovirus LuIII
atcatttttagaactaaccaaccatgttcacgtaagtgacgtgatgacgcgcgctacgcgcgctgccttcggcagtcacacgtcacttacgtctcacatggttggttagttctaaaaatgataagcggttcagggagtttaaaccaaggcgcgaaaaggaagtgggcgtggttttaagtatataagcgacacgttaagtcagttacttactctttcgcttattctgtaagtcgagacacacagagtaaccaactaaccaactagccatggctggaaacgcgtactctgatgaagttttgggaacaactaactggttgaaggataagagcaaccaggaagtattctcatttgtttttaaaaatgaggatgttcagctcaatggaaaaaatatcggatggaacagttacagaaaggagctgcaagaggaggagctgaaatctttacaacgaggagctgaaactacctgggaccagagcgaggacatggaatgggaatcttcagtggatgaactgaccaaaaagcaagtattcatttttgactctttagttaaaaagtgtctctttgaagtactgagcacaaagaacatagctcctagtgatgttacttggtttgtacagcatgaatggggaaaagaccaaggctggcactgtcatgtgctcattggaggcaagaactttagccaggctcaaggaaaatggtggaggagacaattaaatgtttactggagtagatggttggtaacagcctgtagcgtgcagctatcaccagctgaaagaattaaactaagagaaatagcagaagaccaagaatgggttactctgcttacttataagcataagcaaaccaaaaaagactatactaagtgtgtttgctttggaaatatggttgcttactactttttaaccaaaaagaaaatatgtaccagtccaccaagggacggaggctattttctcagtagtgactctggctggaaaactaactttttgaaagaaggcgaacgccatctagtgagcaaactatatactgatgacatgcggccagaaacggttgagaccacagtaaccacagcgcaggaaactaagcgcggcagaattcaaactaagaaggaagtctctattaagactacacttaaagagctggtacataagagagtaacctcaccagaagactggatgatgatgcagccagacagttacattgaaatgatggctcaaccagggggagaaaacctacttaagaatacgctagagatctgtacgctgactctagccagaaccaaaacagcctttgacttgattttagaaaaagctgaaaccagcaaactaaccaactttttactggctgatacaagaacctgtagaatctttgcttttcatggctggaactacatcaaagtctgtcatgctatttgttgtgtcttgaacagacagggaggcaaaagaaatactgttctgtttcatggaccagccagtacaggcaaatcaatcattgcacaggccatagcacaggcagttggtaatgttggttgttataacgcagccaatgtgaactttccatttaatgactgtaccaacaagaacttaatctgggtggaagaagctggtaactttggacagcaagtaaaccagtttaaagccatttgttctggtcagaccattcgcattgaccaaaaaggaaaaggcagcaaacagattgaaccaacaccagtgatcatgaccacaaatgaaaacatcacagtggtcaaaatagggtgtgaagagagaccagaacacactcaaccaatcagagacagaatgttaaacattcatctgacacatacattgcctggtgactttggtttggttgataaaaacgaatggcctatgatatgtgcttggttggtaaagaacggttaccaatcgaccatggcaagttactgtgctaaatggggcaaagttcctgattggacagaaaactgggcggagccaaaagtaacgactgaaataaattcggtaggttcaaccaactcaccatctccgaaaagtacgcctctcagccagaactacgcactaactccgtcggatctcgaggacctggctctggagccttggagcacaccaagtactcctgttgtgggcactgtcaaaaccccgaacactggggaaactggttcaacagcctgtcaagaagctcaacggagcccaacttggtccgagatcgaggaggatttgagagcgtgcttcagttcggaacactggaagagcgactccgaacagctaccaaacttggattaaggtacgatggcgcctccggctaaaagagctaaaagaggtaaggggttaagggatggttggtaggttggtggggtattaatatgtgactacctgttttacaggcctgaaatcacttggttctaggttgggtgcctccaggctacaagtacctgggaccagggaacagccttaaccaaggagaaccaaccaatccatctgacgctgctgctaaagagcacgacgaggcctacgaccaatacatcaaatctggaaagaatccttacctgtacttctctcctgctgatcaacgcttcattgaccaaaccaaagacgctaaagactggggcggaaaggttggtcactacttctttagaaccaagcgtgcttttgcacctaagctttctactgactctgagcctgggacttctggtgtgagcacagctggtaaacgtactaaaccacctgctcacatctttattaaccaagccagggctaaaaaaaaacgtacttctcttgctgcgcagcagaggactcagacaatgagtgatggcaccgaccaatctgacagcggaaacgctgtccagtcagctgctagagttgagcgagcagctgacggtcctggaggctctgggggcgggggctctggtgggggtggggttggcgtttctactggcagttatgataatcaaacacattataagtttctaggggatgggtgggtagagattactgcttacagcacacgcatggtacacttgaacatgcctaaatcagaaaactactgtagggtgcgcgtacacaacacaaatgacacaggtacagcaagtcacatggctatggacgatgctcatgaacagatttggacaccatggagtctggttgatgctaatgcttggggagtttggtttcaaccaagtgactggcagtacatttctaataatatgattcacatcaatttacattcacttgaccaagaattgtttaatgtggtcatcaaaacagtgactgaacagaacacaggagctgaggccattaaggtctacaacaatgacctcactgctgccatgatggttgctcttgattctaacaacatactgccttacacaccagccatagacaatcaagagacacttggtttctatccatggaaaccaaccataccaagtccttacagatactattttagctgtgacagaaacttatcagttacttacaaagacgaagcaggaaccatcactgacacaatgggtttggccagtggcctgaactcccaattttttaccattgagaacactcagcgtattaacctactcagaactggggatgagtatgctactggaacttactactttgacacagaaccaatcagactaactcacacgtggcaaaccaacagacacctgggtcagcctccacaaattactgaactaccaagctctgacactgctaacgctactttaacagctagaggttacagatcaggtctgactcaaattcaaggcagaaatgatgtgactgaagctactagggtcagacctgcacaggttggattttgtcagcctcatgacaattttgaaaccagcagagcggggcctttcaaggttccggtagtgccagcagacatcacacaaggcctagaccatgatgccaatggtagcctgagatatacctatgacaaacaacatggtcaaagctgggcaagtcagaacaacaaagacaggtacacttgggatgctgttaactatgattctggcagatggactaacaactgttttattcaatcagtaccatttacatcagaaccaaatgctaaccaaatacttactaaccgtgacaacctagcgggtaagactgacatacattttaccaacgcatttaacagttatggaccactaactgcttttccacatcctgcgccgatttacccacaagggcagatttgggacaaagaacttgatcttgaacacaagccaagactgcacacacaggctccttttgtctgtaaaaacaatgctccaggtcagcttctggttaggctagcacctaacttgactgaccagtatgatcctaatagttctaacctatctagaattgtcacctatggcaccttcttctggaagggcaaactaactctaaaagcaaagatgagacctaatgctacttggaacccagtcttccaaataagtgctaccaaccaaggaaccaatgactacatgagcattgaaagatggttaccaactgctactggcaacataacaaatgtgcctctgctttctagacctgttgctagaaacacttactaactaactatgctctatgcttcatatatattatatatattattatactaactaaccatgtttactcttacattacttcatataatattaagactaataaaaatacaacatagaaatataatattacatatagatataaagaatagaataatatggtacttacttactgttagaaataatagaacttttggaataacaagatagttagttggtttatgttatatagaatataagaagatgatgtacaaagaataaaagggtgggagggtggttggttggtactcccttagactgaatgttagggaccaaaaaaataataaaattcttgaaaacccaacaaggactactgtcatattcagtgaaccaactgaaccattagtatcaatatgattttagggtgggggggtgggagatacatatgttcactatggaccaactggtactggttggttgctctgctccaaccaaccagaccggctctgccggtctggttggttgagcgcaaccaaccagtaccagttggtccatagtgaacatatgtatctcccacccccccaccctaaaaacatattgatactaatgg

SEQ ID NO: 4 - DNA, 5176 bp, Parvovirus H-1
catttttagaactgaccaaccatgttcacgcaagtgacgtgatgacgcgcgctgcgcgcgctgccttcggcagtcacacgtcactagcgtttcacatggttggtcagttctaaaaatgataagcggttcagagagtttgaaaccaaggcgggaaacggaagtgggcgtggctaactgtatataagcagtcactctggtcggttactcactctgctttcatttctgagtttgtgagacacaggagcgagactaaccaactaaccatggctggaaacgcttactccgatgaggttttgggagtaacaaactggctgaaggacaaaagtagccaggaggtgttctcatttgtttttaaaaatgaaaacgtccaactaaatggaaaggacatcggttggaatagttacagaaaggagctacaagatgacgagctgaagtctctacaacgaggggcggagaccacttgggaccaaagcgaggacatggaatgggagagcgcagtggatgacatgaccaaaaagcaagtatttatttttgattctttggttaagaagtgtttgtttgaagtgctcagcacaaagaacatagctcctagtaatgttacttggttcgtgcagcatgaatggggaaaggacccaggctggcactgtcatgtgctgattggaggcaaggactttagtcaacctcaaggaaaatggtggagaaggcagctaaatgtgtactggagtagatggttggtgactgcctgtaatgttcaactaacaccagctgaaagaattaaactgagagaaatagcagaggacagtgaatgggtcactttgcttacctataagcataagcacaccaagaaggactataccaagtgtgttctttttggaaacatgattgcttattactttttaagcaaaaagaaaatatgtaccagtccaccaagggacggaggctattttcttagcagtgactctggctggaaaactaactttttgaaagagggcgagcgccatctagtgagcaaactgtatactgatgagatgaaaccagaaacggtcgagaccacagtgaccactgcacaggaagctaagcgcggcagaattcaaactagagaggaggtctcgattaaaaccacactcaaagagttggtacataaaagagtaacctcaccagaagactggatgatgatgcagccagacagttacattgaaatgatggctcaaccaggtggagaaaacttgcttaaaaatacactagagatctgtacactgactctagcaagaaccaaaacagcctttgacttgattctggaaaaagctgaaaccagcaaactagccaacttttccatggctagcaccagaacctgtagaatctttgctgagcatggctggaactatattaaagtctgccatgccatctgttgtgtgctgaatagacaaggaggcaaaaggaacactgtgctctttcacggaccagccagcacaggcaaatctattattgcacaagccatagcacaagcagttggtaatgttggttgttacaatgctgccaatgtgaactttccatttaatgactgtaccaacaaaaacttgatttgggtggaagaagctggtaactttggccagcaagtaaaccaattcaaagctatttgttctggccaaaccatacgcattgatcaaaaaggaaaaggcagcaaacagattgaaccaacaccagttattatgaccaccaacgagaacattaccgtggttagaataggctgtgaggaaagaccagaacacactcaaccaatcagagacagaatgctcaacattcacctgacacgtacactacctggtgactttggtttggtggataagcacgaatggcctctgatctgtgcttggttggtgaagaatggttaccaatctaccatggcttgttactgtgctaaatggggcaaagttcctgattggtcagaggactgggcggagccgaagctagacactcctataaattcgctaggttcaatgcgctcaccatctctgactccgagaagtacgcctctcagccaaaactacgctcttactccacttgcatcggaccttgcggacctagctctagagccttggagcacaccaaatactcctgttgcgggcactgcagcaagccaaaacactggggaggctggttccacagcctgccaaggtgctcaacggagcccaacctggtccgagatcgaggcggatttgagagcttgcttcagtcaagaacagttggagagcgacttcaacgaggagctgaccttggactaaggtacaatggcacctccagctaaaagagctaaaagaggtaaggggctaagggatggttggttggtggggtactaatgtatgactacctgttttacaggcctgaaatcacttggttctaggttgggtgcctcctggctacaagtacctgggaccagggaacagccttgaccaaggagaaccaaccaacccttctgacgccgctgccaaagaacacgacgaagcctacgaccaatacatcaaatctggaaaaaatccttacctgtacttctctcctgctgatcaacgcttcattgaccaaaccaaagacgccaaggactggggcggcaaggttggtcactacttttttagaaccaagcgagcttttgcacctaagctttctactgactctgaacctggcacttctggtgtgagcagacctggtaaacgaactaaaccacctgctcacatttttgtaaatcaagccagagctaaaaaaaaacgcgcttctcttgctgcacagcagaggactctgacaatgagtgatggcaccgaaacaaaccaaccagacactggaatcgctaatgctagagttgagcgatcagctgacggaggtggaagctctgggggtgggggctctggcgggggtgggattggtgtttctactgggacttatgataatcaaacgacttataagtttttgggagatggatgggtagaaataactgcacatgcttctagacttttgcacttgggaatgcctccttcagaaaactactgccgcgtcaccgttcacaataatcaaacaacaggacacggaactaaggtaaagggaaacatggcctatgacacacatcaacaaatttggacaccatggagcttggtagatgctaatgcttggggagtttggttccaaccaagtgactggcagttcattcaaaacagcatggaatcgctgaatcttgactcattgagccaagaactatttaatgtagtagtcaaaacagtcactgaacaacaaggagctggccaagatgccattaaagtctataataatgacttgacggcctgtatgatggttgctctggatagtaacaacatactgccttacacacctgcagctcaaacatcagaaacacttggtttctacccatggaaaccaaccgcaccagctccttacagatactactttttcatgcctagacaactcagtgtaacctctagcaactctgctgaaggaactcaaatcacagacaccattggagagccacaggcactaaactctcaattttttactattgagaacaccttgcctattactctcctgcgcacaggtgatgagtttacaactggcacctacatctttaacactgacccacttaaacttactcacacatggcaaaccaacagacacttggcatgcctccaaggaataactgacctaccaacatcagatacagcaacagcatcactaactgcaaatggagacagatttggatcaacacaaacacagaatgtgaactatgtcacagaggctttgcgcaccaggcctgctcagattggcttcatgcaacctcatgacaactttgaagcaaacagaggtggcccatttaaggttccagtggtaccgctagacataacagctggcgaggaccatgatgcaaacggagccatacgatttaactatggcaaacaacatggcgaagattgggccaaacaaggagcagcaccagaaaggtacacatgggatgcaattgatagtgcagctgggagggacacagctagatgctttgtacaaagtgcaccaatatctattccaccaaaccaaaaccagatcttgcagcgagaagacgccatagctggcagaactaacatgcattatactaatgtttttaacagctatggtccacttagtgcatttcctcatccagatcccatttatccaaatggacaaatttgggacaaagaattggacctggaacacaaacctagactacacgtaactgcaccatttgtttgtaaaaacaacccaccaggtcaactatttgttcacttggggcctaatctgactgaccaatttgacccaaacagcacaactgtttctcgcattgttacatatagcactttttactggaagggtattttgaaattcaaagccaaactaagaccaaatctgacctggaatcctgtataccaagcaaccacagactctgttgccaattcttacatgaatgttaagaaatggctcccatctgcaactggcaacatgcactctgatccattgatttgtagacctgtgcctcacatgacatactaaccaaccaactatgtttctctgtttgcttcacataatacttaaactaactagactacaacataaaaatatacacttaataatagattattaaaaataacataatatggtaggttaactgtaaaaaataatagaacttttggaataaatatagttagttggttaatgttagatagaatataaaaagattttgtattttaaaataaatatagttagttggttaatgttagatagaatataaaaagattttgtatttgggaaataaaaagggtggttgggtggttggttggtactcccttagactgaatgttagggaccaaaaaaataataaaataattaaaatgaacaaggactactgtctattcagttgaccaactgaacctatagtatcactatgtttttagggtgggggggtgggagatacatacgttcgctatggaccaagtggtaccggttggttgctaagctcgaacaagacggctaagccggtccggttggttgagcgcaaccaaccggtaccacttggtccatagcgaacgtatgtatctcccacccccccaccctaaaaacatagtgatactataggttcagttggtcaactgaa

SEQ ID NO: 5 - DNA, 21 bp, GS7 (+/+)
gctgctccccccgtggcccct

SEQ ID NO: 6 - DNA, 21 bp, GS7 (+/-)
catcacactggaagactccag

SEQ ID NO: 7 - DNA, 21 bp, GS5 (+/+)
ctgcatgggcggcatgaaccg

SEQ ID NO: 8 - DNA, 21 bp, GS5 (+/-)
cagggctcactccagccacct

SEQ ID NO: 9 - DNA, 15 bp, TP53, NIH3T3, MEF
ggaggtcgtgagacg

SEQ ID NO: 10 - DNA, 15 bp, A9, A9(+/+), A9(+/-)
ggaggtcctgagacg

SEQ ID NO: 11 - DNA, 15 bp, TP53, GS5, GS5(+/+), GS5(+/-),GS7 (+/+)
catgggcggcatgaa

SEQ ID NO: 12 - DNA, 15 bp, GS8, GS9
catgggcagcatgaa

SEQ ID NO: 13 - DNA, 18 bp, Artificial sequence
  Primer forward 34-421
gcagtcagatcctagcgt

SEQ ID NO: 14 - DNA, 18 bp, Artificial sequence
  Primer reverse 34-421
catcttgttgagggcagg

SEQ ID NO: 15 - DNA, 19 bp, Artificial sequence
  Primer forward 301-654
gtcatcttctgtcccttcc

SEQ ID NO: 16 - DNA, 24 bp, Artificial sequence
  Primer reverse 301-654
gtgtttctgtcatccaaatactcc

SEQ ID NO: 17 - DNA, 20 bp, Artificial sequence
  Primer forward 609-990
gagtggaaggaaatttgcgt

SEQ ID NO: 18 - DNA, 21 bp, Artificial sequence
  Primer reverse 609-990
agtggtttcttctttggctgg

SEQ ID NO: 19 - DNA, 19 bp, Artificial sequence
  Primer forward 948-1225
ccaacaacaccagctcctc

SEQ ID NO: 20 - DNA, 24 bp, Artificial sequence
  Primer reverse 948-1225
ggaacaagaagtggagaatgtcag